European Patent Application EP 4 328 240 A1, published February 28, 2024. Title: Recombinant protein production. Applicant: Real Deal Milk S.L. The sequence listing filed with the application follows.

SEQUENCE LISTING (28 sequences)

SEQ ID NO: 1 - protein, 199 aa, Bos taurus
RPKHPIKHQGLPQEVLNENLLRFFVAPFPEVFGKEKVNELSKDIGSESTEDQAMEDIKQMEAESISSSEEIVPNSVEQKHIQKEDVPSERYLGYLEQLLRLKKYKVPQLEIVPNSAEERLHSMKEGIHAQQKEPMIGVNQELAYFYPELFRQFYQLDAYPSGAWYYVPLGTQYTDAPSFSDIPNPIGSENSEKTTMPLW

SEQ ID NO: 2 - protein, 207 aa, Bos taurus
KNTMEHVSSSEESIISQETYKQEKNMAINPSKENLCSTFCKEVVRNANEEEYSIGSSSEESAEVATEEVKITVDDKHYQKALNEINQFYQKFPQYLQYLYQGPIVLNPWDQVKRNAVPITPTLNREQLSTSEENSKKTVDMESTEVFTKKTKLTEEEKNRLNFLKKISQRYQKFALPQYLKTVYQHQKAMKPWIQPKTKVIPYVRYL

SEQ ID NO: 3 - protein, 209 aa, Bos taurus
RELEELNVPGEIVESLSSSEESITRINKKIEKFQSEEQQQTEDELQDKIHPFAQTQSLVYPFPGPIPNSLPQNIPPLTQTPVVVPPFLQPEVMGVSKVKEAMAPKHKEMPFPKYPVEPFTERQSLTLTDVENLHLPLPLLQSWMHQPHQPLPPTVMFPPQSVLSLSQSKVLPVPQKAVPYPQRDMPIQAFLLYQEPVLGPVRGPFPIIV

SEQ ID NO: 4 - protein, 14 aa, Bos taurus
HPHPHLSFMAIPPK

SEQ ID NO: 5 - protein, 27 aa, synthetic construct
  VARIANT 1: note = X is independently selected from A, I, L and V
  VARIANT 4: note = X is independently selected from D and E
  VARIANT 6..8: note = X is independently selected from S and T
  VARIANT 11: note = X is independently selected from A, I, L and V
  VARIANT 12: note = X is independently selected from D and E
  VARIANT 13..14: note = X is independently selected from A, I, L and V
  VARIANT 15: note = X is independently selected from D and E
  VARIANT 17: note = X is independently selected from S and T
  VARIANT 18..19: note = X independently selected from A, I, L and V
  VARIANT 20: note = X is independently selected from S and T
  VARIANT 21: note = X is independently selected from A, I, L and V
  VARIANT 22: note = X is independently selected from D and E
  VARIANT 23: note = X is independently selected from A, I, L and V
  VARIANT 24: note = X is independently selected from S and T
  VARIANT 26: note = X is independently selected from D and E
  VARIANT 27: note = X is independently selected from A, I, L and V
  REGION 1..27: note = CMP fragment
XSGXPXXXPTXXXXXSXXXXXXXXPXX

SEQ ID NO: 6 - protein, 44 aa, synthetic construct
  REGION 1..44: note = CMP fragment
  VARIANT 1: note = X is independently selected from A, I, L and V
  VARIANT 4: note = X is independently selected from D and E
  VARIANT 6..8: note = X is independently selected from S and T
  VARIANT 11: note = X is independently selected from A, I, L and V
  VARIANT 12: note = X is independently selected from D and E
  VARIANT 13..14: note = X is independently selected from A, I, L and V
  VARIANT 15: note = X is independently selected from D and E
  VARIANT 17: note = X is independently selected from S and T
  VARIANT 18..19: note = X is independently selected from A, I, L and V
  VARIANT 20: note = X is independently selected from S and T
  VARIANT 21: note = X is independently selected from A, I, L and V
  VARIANT 22: note = X is independently selected from D and E
  VARIANT 23: note = X is independently selected from A, I, L and V
  VARIANT 24: note = X is independently selected from S and T
  VARIANT 26: note = X is independently selected from D and E
  VARIANT 27..28: note = X is independently selected from A, I, L and V
  VARIANT 29: note = X is independently selected from D and E
  VARIANT 33: note = X is independently selected from D and E
  VARIANT 34: note = X is independently selected from A, I, L and V
  VARIANT 37: note = X is independently selected from A, I, L and V
  VARIANT 39: note = X is independently selected from A, I, L and V
  VARIANT 40: note = X is independently selected from S and T
  VARIANT 43..44: note = X is independently selected from A, I, L and V
XSGXPXXXPTXXXXXSXXXXXXXXPXXXXSPPXXNTXQXXSTXX

SEQ ID NO: 7 - protein, 41 aa, synthetic construct
  REGION 1..41: note = CMP fragment
  VARIANT 4: note = X is independently selected from D and E
  VARIANT 7: note = X is independently selected from D and E
  VARIANT 8: note = X is independently selected from A, I, L and V
  VARIANT 11: note = X is independently selected from A, I, L and V
  VARIANT 14..15: note = X is independently selected from A, I, L and V
  VARIANT 18: note = X is independently selected from D and E
  VARIANT 20..22: note = X is independently selected from S and T
  VARIANT 25: note = X is independently selected from A, I, L and V
  VARIANT 26: note = X is independently selected from D and E
  VARIANT 27..28: note = X is independently selected from A, I, L and V
  VARIANT 29: note = X is independently selected from D and E
  VARIANT 31: note = X is independently selected from S and T
  VARIANT 32..33: note = X is independently selected from A, I, L and V
  VARIANT 34: note = X is independently selected from S and T
  VARIANT 35: note = X is independently selected from A, I, L and V
  VARIANT 36: note = X is independently selected from D and E
  VARIANT 38: note = X is independently selected from S and T
  VARIANT 40: note = X is independently selected from D and E
  VARIANT 41: note = X is independently selected from A, I, L and V
  VARIANT 37: note = X is independently selected from A, I, L and V
  VARIANT 10: note = X is independently selected from S and T
KNQXKTXXPXXNTXXSGXPXXXPTXXXXXSXXXXXXXXPXX

SEQ ID NO: 8 - protein, 58 aa, synthetic construct
  REGION 1..58: note = CMP
  VARIANT 4: note = X is independently selected from D and E
  VARIANT 7: note = X is independently selected from D and E
  VARIANT 8: note = X is independently selected from A, I, L and V
  VARIANT 11: note = X is independently selected from A, I, L and V
  VARIANT 14..15: note = X is independently selected from A, I, L and V
  VARIANT 18: note = X is independently selected from D and E
  VARIANT 20..22: note = X is independently selected from S and T
  VARIANT 25: note = X is independently selected from A, I, L and V
  VARIANT 26: note = X is independently selected from D and E
  VARIANT 27..28: note = X is independently selected from A, I, L and V
  VARIANT 29: note = X is independently selected from D and E
  VARIANT 31: note = X is independently selected from S and T
  VARIANT 32..33: note = X is independently selected from A, I, L and V
  VARIANT 34: note = X is independently selected from S and T
  VARIANT 35: note = X is independently selected from A, I, L and V
  VARIANT 36: note = X is independently selected from D and E
  VARIANT 37: note = X is independently selected from A, I, L and V
  VARIANT 38: note = X is independently selected from S and T
  VARIANT 40: note = X is independently selected from D and E
  VARIANT 41..42: note = X is independently selected from A, I, L and V
  VARIANT 43: note = X is independently selected from D and E
  VARIANT 47: note = X is independently selected from D and E
  VARIANT 48: note = X is independently selected from A, I, L and V
  VARIANT 51: note = X is independently selected from A, I, L and V
  VARIANT 53: note = X is independently selected from A, I, L and V
  VARIANT 54: note = X is independently selected from S and T
  VARIANT 57..58: note = X is independently selected from A, I, L and V
  VARIANT 10: note = X is independently selected from S and T
KNQXKTXXPXXNTXXSGXPXXXPTXXXXXSXXXXXXXXPXXXXSPPXXNTXQXXSTXX

SEQ ID NO: 9 - protein, 27 aa, synthetic construct
  REGION 1..27: note = CMP fragment
ASGEPTSTPTIEAVESTVATLEASPEV

SEQ ID NO: 10 - protein, 44 aa, synthetic construct
  REGION 1..44: note = CMP fragment
ASGEPTSTPTIEAVESTVATLEASPEVIESPPEINTVQVTSTAV

SEQ ID NO: 11 - protein, 41 aa, synthetic construct
  REGION 1..41: note = CMP fragment
KNQDKTEIPTINTIASGEPTSTPTIEAVESTVATLEASPEV

SEQ ID NO: 12 - protein, 58 aa, Bos taurus
KNQDKTEIPTINTIASGEPTSTPTIEAVESTVATLEASPEVIESPPEINTVQVTSTAV

SEQ ID NO: 13 - protein, 8 aa, synthetic construct
  REGION 1..8: note = truncated chymosin cleavage site (bovine)
  VARIANT 5: note = X is L, M or F
HLSFXAIP

SEQ ID NO: 14 - protein, 14 aa, synthetic construct
  REGION 1..14: note = prochymosin cleavage site
  VARIANT 14: note = wherein X is selected from: W, Y, F, C, R, I, M, H, L, V, K, N, T or A
FLQKQQYGISSKFX

SEQ ID NO: 15 - protein, 14 aa, Camelus sp.
RPRPRPSFIAIPPK

SEQ ID NO: 16 - protein, 89 aa, Saccharomyces cerevisiae
MRFPSIFTAVLFAASSALAAPVNTTTEDETAQIPAEAVIGYSDLEGDFDVAVLPFSNSTNNGLLFINTTIASIAAKEEGVSLEKREAEA

SEQ ID NO: 17 - protein, 376 aa, synthetic construct
  REGION 1..376: note = expressed protein as1 casein-CMP (with tags)
MRFPSIFTAVLFAASSALAAPVNTTTEDETAQIPAEAVIGYSDLEGDFDVAVLPFSNSTNNGLLFINTTIASIAAKEEGVSLEKREAEAHHHHHHRPKHPIKHQGLPQEVLNENLLRFFVAPFPEVFGKEKVNELSKDIGSESTEDQAMEDIKQMEAESISSSEEIVPNSVEQKHIQKEDVPSERYLGYLEQLLRLKKYKVPQLEIVPNSAEERLHSMKEGIHAQQKEPMIGVNQELAYFYPELFRQFYQLDAYPSGAWYYVPLGTQYTDAPSFSDIPNPIGSENSEKTTMPLWHPHPHLSFMAIPPKKNQDKTEIPTINTIASGEPTSTPTIEAVESTVATLEASPEVIESPPEINTVQVTSTAVGSGSHHHHHH

SEQ ID NO: 18 - protein, 291 aa, synthetic construct
  REGION 1..291: note = secreted protein as1-CMP (with tags)
EAEAHHHHHHRPKHPIKHQGLPQEVLNENLLRFFVAPFPEVFGKEKVNELSKDIGSESTEDQAMEDIKQMEAESISSSEEIVPNSVEQKHIQKEDVPSERYLGYLEQLLRLKKYKVPQLEIVPNSAEERLHSMKEGIHAQQKEPMIGVNQELAYFYPELFRQFYQLDAYPSGAWYYVPLGTQYTDAPSFSDIPNPIGSENSEKTTMPLWHPHPHLSFMAIPPKKNQDKTEIPTINTIASGEPTSTPTIEAVESTVATLEASPEVIESPPEINTVQVTSTAVGSGSHHHHHH

SEQ ID NO: 19 - protein, 384 aa, synthetic construct
  REGION 1..384: note = expressed protein as2-CMP (with tags)
MRFPSIFTAVLFAASSALAAPVNTTTEDETAQIPAEAVIGYSDLEGDFDVAVLPFSNSTNNGLLFINTTIASIAAKEEGVSLEKREAEAHHHHHHKNTMEHVSSSEESIISQETYKQEKNMAINPSKENLCSTFCKEVVRNANEEEYSIGSSSEESAEVATEEVKITVDDKHYQKALNEINQFYQKFPQYLQYLYQGPIVLNPWDQVKRNAVPITPTLNREQLSTSEENSKKTVDMESTEVFTKKTKLTEEEKNRLNFLKKISQRYQKFALPQYLKTVYQHQKAMKPWIQPKTKVIPYVRYLHPHPHLSFMAIPPKKNQDKTEIPTINTIASGEPTSTPTIEAVESTVATLEASPEVIESPPEINTVQVTSTAVGSGSHHHHHH

SEQ ID NO: 20 - protein, 299 aa, synthetic construct
  REGION 1..299: note = secreted protein as2-CMP
EAEAHHHHHHKNTMEHVSSSEESIISQETYKQEKNMAINPSKENLCSTFCKEVVRNANEEEYSIGSSSEESAEVATEEVKITVDDKHYQKALNEINQFYQKFPQYLQYLYQGPIVLNPWDQVKRNAVPITPTLNREQLSTSEENSKKTVDMESTEVFTKKTKLTEEEKNRLNFLKKISQRYQKFALPQYLKTVYQHQKAMKPWIQPKTKVIPYVRYLHPHPHLSFMAIPPKKNQDKTEIPTINTIASGEPTSTPTIEAVESTVATLEASPEVIESPPEINTVQVTSTAVGSGSHHHHHH

SEQ ID NO: 21 - protein, 386 aa, synthetic construct
  REGION 1..386: note = Expressed protein b casein-CMP
MRFPSIFTAVLFAASSALAAPVNTTTEDETAQIPAEAVIGYSDLEGDFDVAVLPFSNSTNNGLLFINTTIASIAAKEEGVSLEKREAEAHHHHHHRELEELNVPGEIVESLSSSEESITRINKKIEKFQSEEQQQTEDELQDKIHPFAQTQSLVYPFPGPIPNSLPQNIPPLTQTPVVVPPFLQPEVMGVSKVKEAMAPKHKEMPFPKYPVEPFTERQSLTLTDVENLHLPLPLLQSWMHQPHQPLPPTVMFPPQSVLSLSQSKVLPVPQKAVPYPQRDMPIQAFLLYQEPVLGPVRGPFPIIVHPHPHLSFMAIPPKKNQDKTEIPTINTIASGEPTSTPTIEAVESTVATLEASPEVIESPPEINTVQVTSTAVGSGSHHHHHH

SEQ ID NO: 22 - protein, 301 aa, synthetic construct
  REGION 1..301: note = Secreted protein b casein-CMP
EAEAHHHHHHRELEELNVPGEIVESLSSSEESITRINKKIEKFQSEEQQQTEDELQDKIHPFAQTQSLVYPFPGPIPNSLPQNIPPLTQTPVVVPPFLQPEVMGVSKVKEAMAPKHKEMPFPKYPVEPFTERQSLTLTDVENLHLPLPLLQSWMHQPHQPLPPTVMFPPQSVLSLSQSKVLPVPQKAVPYPQRDMPIQAFLLYQEPVLGPVRGPFPIIVHPHPHLSFMAIPPKKNQDKTEIPTINTIASGEPTSTPTIEAVESTVATLEASPEVIESPPEINTVQVTSTAVGSGSHHHHHH

SEQ ID NO: 23 - DNA, 1131 bp, synthetic construct
  source 1..1131: mol_type = other DNA
  misc_feature 1..1131: note = DNA encoding expressed protein as1 casein-CMP (with tags)
atgagatttccatctattttcactgctgttttgtttgctgcttcttctgctttggctgctccagttaacactactactgaagatgagactgctcaaattcctgctgaagctgttattggttactctgatttggagggagattttgatgttgctgttttgcctttctctaactctactaacaacggtttgttgttcattaacactactatcgcttctatcgctgctaaggaagagggtgtttctttggaaaagagagaagctgaggctcaccatcaccaccatcacagaccaaagcatcctattaaacaccaaggtttgccacaagaagttttgaacgagaatttgttgagatttttcgttgctccatttcctgaagttttcggtaaagaaaaagttaacgagttgtctaaggatattggttctgaatctactgaggatcaagctatggaagatatcaagcaaatggaagctgagtctatctcttcttctgaagagattgttccaaactctgttgaacaaaagcatatccaaaaggaagatgttccttctgagagatacttgggttatttggaacaattgttgagattgaagaaatacaaggttccacaattggagattgttcctaactctgctgaagagagattgcattctatgaaggaaggtattcacgctcaacaaaaagagccaatgattggtgttaatcaagaattggcttacttctaccctgagttgtttagacaattctaccaattggatgcttatccatctggtgcttggtactatgttcctttgggtactcaatacactgatgctccatctttctctgatattccaaaccctattggttctgaaaattctgagaaaactactatgcctttgtggcatccacaccctcatttgtctttcatggctattccacctaagaaaaaccaagataagactgaaatcccaactattaatactattgcttctggagagccaacttctactcctactattgaagctgttgagtctactgttgctactttggaagcttctcctgaagttattgagtctccacctgagattaatactgttcaagttacttctactgctgttggttctggatcccatcaccatcaccatcactaa

SEQ ID NO: 24 - DNA, 1155 bp, synthetic construct
  source 1..1155: mol_type = other DNA
  misc_feature 1..1155: note = DNA encoding expressed protein as2-CMP
atgagatttccatctattttcactgctgttttgtttgctgcttcttctgctttggctgctccagttaacactactactgaagatgagactgctcaaattcctgctgaagctgttattggttactctgatttggagggagattttgatgttgctgttttgcctttctctaactctactaacaacggtttgttgttcattaacactactatcgcttctatcgctgctaaggaagagggtgtttctttggaaaagagagaagctgaggctcaccatcaccaccatcacaagaacactatggaacatgtttcttcttctgaagagtctatcatctctcaagaaacttacaagcaagagaaaaacatggctattaatccatctaaggaaaatttgtgttctactttctgtaaggaggttgttagaaacgctaatgaagaggaatactctattggttcttcttctgaggaatctgctgaagttgctactgaggaagttaagatcactgttgatgataagcactaccaaaaggctttgaacgagattaatcaattctaccaaaagttccctcaatatttgcaatacttgtatcaaggtccaattgttttgaacccttgggatcaagttaagagaaacgctgttccaatcactcctactttgaacagagaacaattgtctacttctgaggaaaactctaagaaaactgttgatatggaatctactgaggtttttactaagaaaactaagttgactgaggaagagaaaaacagattgaactttttgaagaagatttctcaaagataccaaaagttcgctttgccacaatacttgaagactgtttaccaacatcaaaaggctatgaaaccatggattcaacctaagactaaagttattccttacgttagatatttgcatccacaccctcatttgtctttcatggctattccacctaagaaaaaccaagataagactgaaatcccaactattaatactattgcttctggagagccaacttctactcctactattgaagctgttgagtctactgttgctactttggaagcttctcctgaagttattgagtctccacctgagattaatactgttcaagttacttctactgctgttggttctggatcccatcaccatcaccatcactaa

SEQ ID NO: 25 - DNA, 1161 bp, synthetic construct
  source 1..1161: mol_type = other DNA
  misc_feature 1..1161: note = DNA encoding Expressed protein b casein-CMP (with tags)
atgagatttccatctattttcactgctgttttgtttgctgcttcttctgctttggctgctccagttaacactactactgaagatgagactgctcaaattcctgctgaagctgttattggttactctgatttggagggagattttgatgttgctgttttgcctttctctaactctactaacaacggtttgttgttcattaacactactatcgcttctatcgctgctaaggaagagggtgtttctttggaaaagagagaagctgaggctcaccatcaccaccatcacagagaattggaagagttgaacgttccaggtgaaattgttgagtctttgtcttcttctgaagagtctatcactagaattaataagaaaattgagaagtttcaatctgaagagcaacaacaaactgaagatgagttgcaagataagatccatccattcgctcaaactcaatctttggtttacccattccctggtccaattcctaactctttgcctcaaaatattccacctttgactcaaactccagttgttgttccacctttcttgcaacctgaagttatgggtgtttctaaggttaaagaagctatggctccaaagcataaagagatgccatttcctaagtatccagttgaacctttcactgagagacaatctttgactttgactgatgttgaaaacttgcacttgccattgcctttgttgcaatcttggatgcatcaaccacaccaacctttgccacctactgttatgtttccacctcaatctgttttgtctttgtctcaatctaaggttttgccagttcctcaaaaagctgttccataccctcaaagagatatgccaattcaagctttcttgttgtatcaagaaccagttttgggtcctgttagaggtccatttcctattattgttcatccacaccctcatttgtctttcatggctattccacctaagaaaaaccaagataagactgaaatcccaactattaatactattgcttctggagagccaacttctactcctactattgaagctgttgagtctactgttgctactttggaagcttctcctgaagttattgagtctccacctgagattaatactgttcaagttacttctactgctgttggttctggatcccatcaccatcaccatcactaa

SEQ ID NO: 26 - protein, 217 aa, synthetic construct
  REGION 1..217: note = Recombinant as1 casein
EAEAHHHHHHRPKHPIKHQGLPQEVLNENLLRFFVAPFPEVFGKEKVNELSKDIGSESTEDQAMEDIKQMEAESISSSEEIVPNSVEQKHIQKEDVPSERYLGYLEQLLRLKKYKVPQLEIVPNSAEERLHSMKEGIHAQQKEPMIGVNQELAYFYPELFRQFYQLDAYPSGAWYYVPLGTQYTDAPSFSDIPNPIGSENSEKTTMPLWHPHPHLSF

SEQ ID NO: 27 - protein, 225 aa, synthetic construct
  REGION 1..225: note = Recombinant as2 casein
EAEAHHHHHHKNTMEHVSSSEESIISQETYKQEKNMAINPSKENLCSTFCKEVVRNANEEEYSIGSSSEESAEVATEEVKITVDDKHYQKALNEINQFYQKFPQYLQYLYQGPIVLNPWDQVKRNAVPITPTLNREQLSTSEENSKKTVDMESTEVFTKKTKLTEEEKNRLNFLKKISQRYQKFALPQYLKTVYQHQKAMKPWIQPKTKVIPYVRYLHPHPHLSF

SEQ ID NO: 28 - protein, 227 aa, synthetic construct
  REGION 1..227: note = Recombinant b casein
EAEAHHHHHHRELEELNVPGEIVESLSSSEESITRINKKIEKFQSEEQQQTEDELQDKIHPFAQTQSLVYPFPGPIPNSLPQNIPPLTQTPVVVPPFLQPEVMGVSKVKEAMAPKHKEMPFPKYPVEPFTERQSLTLTDVENLHLPLPLLQSWMHQPHQPLPPTVMFPPQSVLSLSQSKVLPVPQKAVPYPQRDMPIQAFLLYQEPVLGPVRGPFPIIVHPHPHLSF